European Patent Application EP 4 717 704 A1, published April 1, 2026. Title: Novel Protein A ligand that enables milder elution. Applicant: Cytiva BioProcess R&D AB. The sequence listing filed with the application follows.

SEQUENCE LISTING (54 sequences)

SEQ ID NO: 1 - protein, 58 aa, Staphylococcus aureus
ADNKFNKEQQNAFYEILHLPNLTEEQRNGFIQSLKDDPSVSKEILAEAKKLNDAQAPK

SEQ ID NO: 2 - protein, 58 aa, Staphylococcus aureus [sequence omitted]

SEQ ID NO: 3 - protein, 58 aa, Staphylococcus aureus
ADNNFNKEQQNAFYEILNMPNLNEEQRNGFIQSLKDDPSQSANLLAEAKKLNESQAPK

SEQ ID NO: 4 - protein, 61 aa, Staphylococcus aureus
ADAQQNKFNKDQQSAFYEILNMPNLNEEQRNGFIQSLKDDPSQSTNVLGEAKKLNESQAPK

SEQ ID NO: 5 - protein, 56 aa, Staphylococcus aureus
AQHDEAQQNAFYQVLNMPNLNADQRNGFIQSLKDDPSQSANVLGEAQKLNDSQAPK

SEQ ID NO: 6 - protein, 58 aa, synthetic construct [sequence omitted]

SEQ ID NO: 7 - protein, 58 aa, synthetic construct [sequence omitted]

SEQ ID NO: 8 - protein, 58 aa, synthetic construct
VDAKFDKEAQEAFYEILHLPNLTEEQRNAFIQSLKDDPSGSKAILAEAKKVNDAQAPK

SEQ ID NO: 9 - protein, 58 aa, synthetic construct
VDAKFDKEAQEAFYEILHLPNLTEEQRNAFIQSLKDDPSVSKAILAEAKKLNDAQAPK

SEQ ID NO: 10 - protein, 58 aa, synthetic construct
VDAKFDKEQQNAFYEILSLPNLTEEQRAAFIQSLKDDPSQSANLLAEAKKLNDAQAPK

SEQ ID NO: 11 - protein, 58 aa, synthetic construct
VDAKFDKEQQNAFYEILHLPNLTEEQRNAFIQSLKDDPSGSKAILAEAKKVNDAQAPK

SEQ ID NO: 12 - protein, 11 aa, synthetic construct
  VARIANT 1: note = X in position 1 is R or K
  VARIANT 7: note = X in position 7 is H or D or Q or E
  VARIANT 11: note = X in position 11 is H or T or K or S or G
XLPNLTXEQRX

SEQ ID NO: 13 - protein, 34 aa, synthetic construct
  VARIANT 1: note = X in position 1 is R or K
  VARIANT 7: note = X in position 7 is H or D or Q or E
  VARIANT 11: note = X in position 11 is H or T or K or S or G
  VARIANT 12: note = X in position 12 is A or G
  VARIANT 16: note = X in position 16 is T or S or G or Q or A or E or H or R or P or D or K or N
  VARIANT 18: note = X in position 18 is R or K
  VARIANT 23: note = X in position 23 is V or E or G or R or D or K or Q or N or H or S
  VARIANT 25: note = X in position 25 is K or A or T
  VARIANT 26: note = X in position 26 is N or A or E
  VARIANT 27: note = X in position 27 is I or L or V
  VARIANT 29: note = X in position 29 is A or G
  VARIANT 32: note = X in position 32 is K or Q
  VARIANT 34: note = X in position 34 is L or V or S or I or R or G
XLPNLTXEQRXXFIQXLXDDPSXSXXXLXEAXKX

SEQ ID NO: 14 - protein, 20 aa, synthetic construct
  VARIANT 1: note = X in position 1 is A or Q
  VARIANT 3: note = X in position 3 is E or N or H or R or S
  VARIANT 7: note = X in position 7 is E or Q or H
  VARIANT 8: note = X in position 8 is I or V
  VARIANT 10: note = X in position 10 is R or K
  VARIANT 16: note = X in position 16 is H or D or Q or E
  VARIANT 20: note = X in position 20 is H or T or K or S or G
XQXAFYXXLXLPNLTXEQRX

SEQ ID NO: 15 - protein, 43 aa, synthetic construct
  VARIANT 1: note = X in position 1 is A or Q
  VARIANT 3: note = X in position 3 is E or N or H or R or S
  VARIANT 7: note = X in position 7 is E or Q or H
  VARIANT 8: note = X in position 8 is I or V
  VARIANT 10: note = X in position 10 is R or K
  VARIANT 16: note = X in position 16 is H or D or Q or E
  VARIANT 20: note = X in position 20 is H or T or K or S or G
  VARIANT 21: note = X in position 21 is A or G
  VARIANT 25: note = X in position 25 is T or S or G or Q or A or E or H or R or P or D or K or N
  VARIANT 27: note = X in position 27 is R or K
  VARIANT 32: note = X in position 32 is V or E or G or R or D or K or Q or N or H or S
  VARIANT 34: note = X in position 34 is K or A or T
  VARIANT 35: note = X in position 35 is N or A or E
  VARIANT 36: note = X in position 36 is I or L or V
  VARIANT 38: note = X in position 38 is A or G
  VARIANT 41: note = X in position 41 is K or Q
  VARIANT 43: note = X in position 43 is L or V or S or I or R or G
XQXAFYXXLXLPNLTXEQRXXFIQXLXDDPSXSXXXLXEAXKX

SEQ ID NO: 16 - protein, 58 aa, synthetic construct
VDAKFDKEQQNAFYEILKLPNLTDEQRTAFIQSLKDDPSGSKAILAEAKKVNDAQAPK

SEQ ID NO: 17 - protein, 58 aa, synthetic construct
VDAKFDKEQQNAFYEILKLPNLTQEQRTAFIQSLKDDPSGSKAILAEAKKVNDAQAPK

SEQ ID NO: 18 - protein, 58 aa, synthetic construct
VDAKFDKEQQNAFYEILRLPNLTHEQRGAFIQSLKDDPSGSKAILAEAKKVNDAQAPK

SEQ ID NO: 19 - protein, 58 aa, synthetic construct
VDAKFDKEQQNAFYEILRLPNLTDEQRGAFIQSLKDDPSGSKAILAEAKKVNDAQAPK

SEQ ID NO: 20 - protein, 58 aa, synthetic construct
VDAKFDKEQQNAFYEILRLPNLTDEQRKAFIQSLKDDPSGSKAILAEAKKVNDAQAPK

SEQ ID NO: 21 - protein, 58 aa, synthetic construct
VDAKFDKEQQNAFYEILRLPNLTEEQRSAFIQSLKDDPSGSKAILAEAKKVNDAQAPK

SEQ ID NO: 22 - protein, 58 aa, synthetic construct
VDAKFDKEQQNAFYEILKLPNLTDEQRGAFIQSLKDDPSGSKAILAEAKKVNDAQAPK

SEQ ID NO: 23 - protein, 58 aa, synthetic construct
VDAKFDKEQQNAFYEILKLPNLTHEQRTAFIQSLKDDPSGSKAILAEAKKVNDAQAPK

SEQ ID NO: 24 - protein, 58 aa, synthetic construct
VDAKFDKEQQNAFYEILRLPNLTHEQRSAFIQSLKDDPSGSKAILAEAKKVNDAQAPK

SEQ ID NO: 25 - protein, 58 aa, synthetic construct
VDAKFDKEQQNAFYEILKLPNLTHEQRGAFIQSLKDDPSGSKAILAEAKKVNDAQAPK

SEQ ID NO: 26 - protein, 58 aa, synthetic construct
VDAKFDKEQQNAFYEILRLPNLTHEQRHAFIQSLKDDPSGSKAILAEAKKVNDAQAPK

SEQ ID NO: 27 - protein, 58 aa, synthetic construct
VDAKFDKEAQNAFYEILRLPNLTHEQRGAFIQSLKDDPSGSKAILAEAKKVNDAQAPK

SEQ ID NO: 28 - protein, 58 aa, synthetic construct
VDAKFDKEQQEAFYEILRLPNLTHEQRGAFIQSLKDDPSGSKAILAEAKKVNDAQAPK

SEQ ID NO: 29 - protein, 58 aa, synthetic construct
VDAKFDKEQQHAFYEILRLPNLTHEQRGAFIQSLKDDPSGSKAILAEAKKVNDAQAPK

SEQ ID NO: 30 - protein, 58 aa, synthetic construct
VDAKFDKEAQEAFYEILRLPNLTHEQRGAFIQSLKDDPSGSKAILAEAKKVNDAQAPK

SEQ ID NO: 31 - protein, 58 aa, synthetic construct
VDAKFDKEQQEAFYEILRLPNLTHEQRHAFIQSLKDDPSGSKAILAEAKKVNDAQAPK

SEQ ID NO: 32 - protein, 58 aa, synthetic construct
VDAKFDKEQQRAFYEILRLPNLTHEQRHAFIQSLKDDPSGSKAILAEAKKVNDAQAPK

SEQ ID NO: 33 - protein, 58 aa, synthetic construct
VDAKFDKEQQNAFYHILRLPNLTHEQRGAFIQSLKDDPSGSKAILAEAKKVNDAQAPK

SEQ ID NO: 34 - protein, 131 aa, synthetic construct
AQYEDGKQYTGTVDAKFDKEQQNAFYEILSLPNLTEEQRAAFIQSLKDDPSQSANLLAEAKKLNDAQAPKASGGGSLAEAKVLANRELDKYGVSDYYKNLINNAKTVEGVKALIDEILAALPKASHHHHHH

SEQ ID NO: 35 - protein, 131 aa, synthetic construct
AQYEDGKQYTGTVDAKFDKEQQNAFYEILKLPNLTDEQRTAFIQSLKDDPSGSKAILAEAKKVNDAQAPKASGGGSLAEAKVLANRELDKYGVSDYYKNLINNAKTVEGVKALIDEILAALPKASHHHHHH

SEQ ID NO: 36 - protein, 131 aa, synthetic construct
AQYEDGKQYTGTVDAKFDKEQQNAFYEILKLPNLTQEQRTAFIQSLKDDPSGSKAILAEAKKVNDAQAPKASGGGSLAEAKVLANRELDKYGVSDYYKNLINNAKTVEGVKALIDEILAALPKASHHHHHH

SEQ ID NO: 37 - protein, 131 aa, synthetic construct
AQYEDGKQYTGTVDAKFDKEQQNAFYEILRLPNLTHEQRGAFIQSLKDDPSGSKAILAEAKKVNDAQAPKASGGGSLAEAKVLANRELDKYGVSDYYKNLINNAKTVEGVKALIDEILAALPKASHHHHHH

SEQ ID NO: 38 - protein, 131 aa, synthetic construct
AQYEDGKQYTGTVDAKFDKEQQNAFYEILRLPNLTDEQRGAFIQSLKDDPSGSKAILAEAKKVNDAQAPKASGGGSLAEAKVLANRELDKYGVSDYYKNLINNAKTVEGVKALIDEILAALPKASHHHHHH

SEQ ID NO: 39 - protein, 131 aa, synthetic construct
AQYEDGKQYTGTVDAKFDKEQQNAFYEILRLPNLTDEQRKAFIQSLKDDPSGSKAILAEAKKVNDAQAPKASGGGSLAEAKVLANRELDKYGVSDYYKNLINNAKTVEGVKALIDEILAALPKASHHHHHH

SEQ ID NO: 40 - protein, 131 aa, synthetic construct
AQYEDGKQYTGTVDAKFDKEQQNAFYEILRLPNLTEEQRSAFIQSLKDDPSGSKAILAEAKKVNDAQAPKASGGGSLAEAKVLANRELDKYGVSDYYKNLINNAKTVEGVKALIDEILAALPKASHHHHHH

SEQ ID NO: 41 - protein, 131 aa, synthetic construct
AQYEDGKQYTGTVDAKFDKEQQNAFYEILKLPNLTDEQRGAFIQSLKDDPSGSKAILAEAKKVNDAQAPKASGGGSLAEAKVLANRELDKYGVSDYYKNLINNAKTVEGVKALIDEILAALPKASHHHHHH

SEQ ID NO: 42 - protein, 12 aa, synthetic construct
AQYEDGKQYTGT

SEQ ID NO: 43 - protein, 12 aa, synthetic construct
AQYEDGKQYTDT

SEQ ID NO: 44 - protein, 61 aa, synthetic construct
ASGGGSLAEAKVLANRELDKYGVSDYYKNLINNAKTVEGVKALIDEILAALPKASHHHHHH

SEQ ID NO: 45 - protein, 348 aa, synthetic construct
VDAKFDKEQQEAFYEILRLPNLTHEQRHAFIQSLKDDPSGSKAILAEAKKVNDAQAPKVDAKFDKEQQEAFYEILRLPNLTHEQRHAFIQSLKDDPSGSKAILAEAKKVNDAQAPKVDAKFDKEQQEAFYEILRLPNLTHEQRHAFIQSLKDDPSGSKAILAEAKKVNDAQAPKVDAKFDKEQQEAFYEILRLPNLTHEQRHAFIQSLKDDPSGSKAILAEAKKVNDAQAPKVDAKFDKEQQEAFYEILRLPNLTHEQRHAFIQSLKDDPSGSKAILAEAKKVNDAQAPKVDAKFDKEQQEAFYEILRLPNLTHEQRHAFIQSLKDDPSGSKAILAEAKKVNDAQAPK

SEQ ID NO: 46 - protein, 348 aa, synthetic construct
VDAKFDKEQQNAFYEILRLPNLTHEQRHAFIQSLKDDPSGSKAILAEAKKVNDAQAPKVDAKFDKEQQNAFYEILRLPNLTHEQRHAFIQSLKDDPSGSKAILAEAKKVNDAQAPKVDAKFDKEQQNAFYEILRLPNLTHEQRHAFIQSLKDDPSGSKAILAEAKKVNDAQAPKVDAKFDKEQQNAFYEILRLPNLTHEQRHAFIQSLKDDPSGSKAILAEAKKVNDAQAPKVDAKFDKEQQNAFYEILRLPNLTHEQRHAFIQSLKDDPSGSKAILAEAKKVNDAQAPKVDAKFDKEQQNAFYEILRLPNLTHEQRHAFIQSLKDDPSGSKAILAEAKKVNDAQAPK

SEQ ID NO: 47 - protein, 348 aa, synthetic construct
VDAKFDKEQQEAFYEILRLPNLTHEQRGAFIQSLKDDPSGSKAILAEAKKVNDAQAPKVDAKFDKEQQEAFYEILRLPNLTHEQRGAFIQSLKDDPSGSKAILAEAKKVNDAQAPKVDAKFDKEQQEAFYEILRLPNLTHEQRGAFIQSLKDDPSGSKAILAEAKKVNDAQAPKVDAKFDKEQQEAFYEILRLPNLTHEQRGAFIQSLKDDPSGSKAILAEAKKVNDAQAPKVDAKFDKEQQEAFYEILRLPNLTHEQRGAFIQSLKDDPSGSKAILAEAKKVNDAQAPKVDAKFDKEQQEAFYEILRLPNLTHEQRGAFIQSLKDDPSGSKAILAEAKKVNDAQAPK

SEQ ID NO: 48 - protein, 348 aa, synthetic construct
VDAKFDKEQQNAFYEILRLPNLTHEQRGAFIQSLKDDPSGSKAILAEAKKVNDAQAPKVDAKFDKEQQNAFYEILRLPNLTHEQRGAFIQSLKDDPSGSKAILAEAKKVNDAQAPKVDAKFDKEQQNAFYEILRLPNLTHEQRGAFIQSLKDDPSGSKAILAEAKKVNDAQAPKVDAKFDKEQQNAFYEILRLPNLTHEQRGAFIQSLKDDPSGSKAILAEAKKVNDAQAPKVDAKFDKEQQNAFYEILRLPNLTHEQRGAFIQSLKDDPSGSKAILAEAKKVNDAQAPKVDAKFDKEQQNAFYEILRLPNLTHEQRGAFIQSLKDDPSGSKAILAEAKKVNDAQAPK

SEQ ID NO: 49 - protein, 348 aa, synthetic construct
VDAKFDKEAQNAFYEILRLPNLTHEQRGAFIQSLKDDPSGSKAILAEAKKVNDAQAPKVDAKFDKEAQNAFYEILRLPNLTHEQRGAFIQSLKDDPSGSKAILAEAKKVNDAQAPKVDAKFDKEAQNAFYEILRLPNLTHEQRGAFIQSLKDDPSGSKAILAEAKKVNDAQAPKVDAKFDKEAQNAFYEILRLPNLTHEQRGAFIQSLKDDPSGSKAILAEAKKVNDAQAPKVDAKFDKEAQNAFYEILRLPNLTHEQRGAFIQSLKDDPSGSKAILAEAKKVNDAQAPKVDAKFDKEAQNAFYEILRLPNLTHEQRGAFIQSLKDDPSGSKAILAEAKKVNDAQAPK

SEQ ID NO: 50 - protein, 361 aa, synthetic construct
AQYEDGKQYTDTVDAKFDKEQQEAFYEILRLPNLTHEQRHAFIQSLKDDPSGSKAILAEAKKVNDAQAPKVDAKFDKEQQEAFYEILRLPNLTHEQRHAFIQSLKDDPSGSKAILAEAKKVNDAQAPKVDAKFDKEQQEAFYEILRLPNLTHEQRHAFIQSLKDDPSGSKAILAEAKKVNDAQAPKVDAKFDKEQQEAFYEILRLPNLTHEQRHAFIQSLKDDPSGSKAILAEAKKVNDAQAPKVDAKFDKEQQEAFYEILRLPNLTHEQRHAFIQSLKDDPSGSKAILAEAKKVNDAQAPKVDAKFDKEQQEAFYEILRLPNLTHEQRHAFIQSLKDDPSGSKAILAEAKKVNDAQAPKC

SEQ ID NO: 51 - protein, 361 aa, synthetic construct
AQYEDGKQYTDTVDAKFDKEQQNAFYEILRLPNLTHEQRHAFIQSLKDDPSGSKAILAEAKKVNDAQAPKVDAKFDKEQQNAFYEILRLPNLTHEQRHAFIQSLKDDPSGSKAILAEAKKVNDAQAPKVDAKFDKEQQNAFYEILRLPNLTHEQRHAFIQSLKDDPSGSKAILAEAKKVNDAQAPKVDAKFDKEQQNAFYEILRLPNLTHEQRHAFIQSLKDDPSGSKAILAEAKKVNDAQAPKVDAKFDKEQQNAFYEILRLPNLTHEQRHAFIQSLKDDPSGSKAILAEAKKVNDAQAPKVDAKFDKEQQNAFYEILRLPNLTHEQRHAFIQSLKDDPSGSKAILAEAKKVNDAQAPKC

SEQ ID NO: 52 - protein, 361 aa, synthetic construct
AQYEDGKQYTDTVDAKFDKEQQEAFYEILRLPNLTHEQRGAFIQSLKDDPSGSKAILAEAKKVNDAQAPKVDAKFDKEQQEAFYEILRLPNLTHEQRGAFIQSLKDDPSGSKAILAEAKKVNDAQAPKVDAKFDKEQQEAFYEILRLPNLTHEQRGAFIQSLKDDPSGSKAILAEAKKVNDAQAPKVDAKFDKEQQEAFYEILRLPNLTHEQRGAFIQSLKDDPSGSKAILAEAKKVNDAQAPKVDAKFDKEQQEAFYEILRLPNLTHEQRGAFIQSLKDDPSGSKAILAEAKKVNDAQAPKVDAKFDKEQQEAFYEILRLPNLTHEQRGAFIQSLKDDPSGSKAILAEAKKVNDAQAPKC

SEQ ID NO: 53 - protein, 361 aa, synthetic construct
AQYEDGKQYTDTVDAKFDKEQQNAFYEILRLPNLTHEQRGAFIQSLKDDPSGSKAILAEAKKVNDAQAPKVDAKFDKEQQNAFYEILRLPNLTHEQRGAFIQSLKDDPSGSKAILAEAKKVNDAQAPKVDAKFDKEQQNAFYEILRLPNLTHEQRGAFIQSLKDDPSGSKAILAEAKKVNDAQAPKVDAKFDKEQQNAFYEILRLPNLTHEQRGAFIQSLKDDPSGSKAILAEAKKVNDAQAPKVDAKFDKEQQNAFYEILRLPNLTHEQRGAFIQSLKDDPSGSKAILAEAKKVNDAQAPKVDAKFDKEQQNAFYEILRLPNLTHEQRGAFIQSLKDDPSGSKAILAEAKKVNDAQAPKC

SEQ ID NO: 54 - protein, 361 aa, synthetic construct
AQYEDGKQYTDTVDAKFDKEAQNAFYEILRLPNLTHEQRGAFIQSLKDDPSGSKAILAEAKKVNDAQAPKVDAKFDKEAQNAFYEILRLPNLTHEQRGAFIQSLKDDPSGSKAILAEAKKVNDAQAPKVDAKFDKEAQNAFYEILRLPNLTHEQRGAFIQSLKDDPSGSKAILAEAKKVNDAQAPKVDAKFDKEAQNAFYEILRLPNLTHEQRGAFIQSLKDDPSGSKAILAEAKKVNDAQAPKVDAKFDKEAQNAFYEILRLPNLTHEQRGAFIQSLKDDPSGSKAILAEAKKVNDAQAPKVDAKFDKEAQNAFYEILRLPNLTHEQRGAFIQSLKDDPSGSKAILAEAKKVNDAQAPKC